European Patent Specification EP 3 718 566 B1, published June 12, 2024. Title: Modified RSV F Proteins and Methods of Their Use. Applicant: Novavax, Inc. The sequence listing filed with the application follows.

SEQUENCE LISTING (29 sequences)

SEQ ID NO: 1 - DNA, 1725 bp, respiratory syncytial virus
atggagttgctaatcctcaaagcaaatgcaattaccacaatcctcactgcagtcacattttgttttgcttctggtcaaaacatcactgaagaattttatcaatcaacatgcagtgcagttagcaaaggctatcttagtgctctgagaactggttggtataccagtgttataactatagaattaagtaatatcaaggaaaataagtgtaatggaacagatgctaaggtaaaattgataaaacaagaattagataaatataaaaatgctgtaacagaattgcagttgctcatgcaaagcacaccaccaacaaacaatcgagccagaagagaactaccaaggtttatgaattatacactcaacaatgccaaaaaaaccaatgtaacattaagcaagaaaaggaaaagaagatttcttggttttttgttaggtgttggatctgcaatcgccagtggcgttgctgtatctaaggtcctgcacctagaaggggaagtgaacaagatcaaaagtgctctactatccacaaacaaggctgtagtcagcttatcaaatggagttagtgtcttaaccagcaaagtgttagacctcaaaaactatatagataaacaattgttacctattgtgaacaagcaaagctgcagcatatcaaatatagaaactgtgatagagttccaacaaaagaacaacagactactagagattaccagggaatttagtgttaatgcaggtgtaactacacctgtaagcacttacatgttaactaatagtgaattattgtcattaatcaatgatatgcctataacaaatgatcagaaaaagttaatgtccaacaatgttcaaatagttagacagcaaagttactctatcatgtccataataaaagaggaagtcttagcatatgtagtacaattaccactatatggtgttatagatacaccctgttggaaactacacacatcccctctatgtacaaccaacacaaaagaagggtccaacatctgtttaacaagaactgacagaggatggtactgtgacaatgcaggatcagtatctttcttcccacaagctgaaacatgtaaagttcaatcaaatcgagtattttgtgacacaatgaacagtttaacattaccaagtgaaataaatctctgcaatgttgacatattcaaccccaaatatgattgtaaaattatgacttcaaaaacagatgtaagcagctccgttatcacatctctaggagccattgtgtcatgctatggcaaaactaaatgtacagcatccaataaaaatcgtggaatcataaagacattttctaacgggtgcgattatgtatcaaataaagggatggacactgtgtctgtaggtaacacattatattatgtaaataagcaagaaggtaaaagtctctatgtaaaaggtgaaccaataataaatttctatgacccattagtattcccctctgatgaatttgatgcatcaatatctcaagtcaacgagaagattaaccagagcctagcatttattcgtaaatccgatgaattattacataatgtaaatgctggtaaatccaccacaaatatcatgataactactataattatagtgattatagtaatattgttatcattaattgctgttggactgctcttatactgtaaggccagaagcacaccagtcacactaagcaaagatcaactgagtggtataaataatattgcatttagtaactaa

SEQ ID NO: 2 - protein, 574 aa, respiratory syncytial virus
MELLILKANAITTILTAVTFCFASGQNITEEFYQSTCSAVSKGYLSALRTGWYTSVITIELSNIKENKCNGTDAKVKLIKQELDKYKNAVTELQLLMQSTPPTNNRARRELPRFMNYTLNNAKKTNVTLSKKRKRRFLGFLLGVGSAIASGVAVSKVLHLEGEVNKIKSALLSTNKAVVSLSNGVSVLTSKVLDLKNYIDKQLLPIVNKQSCSISNIETVIEFQQKNNRLLEITREFSVNAGVTTPVSTYMLTNSELLSLINDMPITNDQKKLMSNNVQIVRQQSYSIMSIIKEEVLAYVVQLPLYGVIDTPCWKLHTSPLCTTNTKEGSNICLTRTDRGWYCDNAGSVSFFPQAETCKVQSNRVFCDTMNSLTLPSEINLCNVDIFNPKYDCKIMTSKTDVSSSVITSLGAIVSCYGKTKCTASNKNRGIIKTFSNGCDYVSNKGMDTVSVGNTLYYVNKQEGKSLYVKGEPIINFYDPLVFPSDEFDASISQVNEKINQSLAFIRKSDELLHNVNAGKSTTNIMITTIIIVIIVILLSLIAVGLLLYCKARSTPVTLSKDQLSGINNIAFSN

SEQ ID NO: 3 - DNA, 1725 bp, Artificial Sequence
  F Protein 576
atggagctgctcatcttgaaggctaacgccattaccactatccttacagcggtgacgttctgctttgcatccggtcagaatattaccgaagagttctaccaatctacttgtagcgctgtctcaaaaggctatctgtcggccctccgtacaggatggtacacgagtgttatcaccatcgaattgtccaacattaaggagaacaagtgcaacggtactgacgcgaaggtaaagcttatcaaacaggaactggataagtacaagaacgcagtgacagagctccaattgctgatgcagtctacccccgctacgaataaccgcgctaggagagaacttccacgattcatgaactatactctcaataacgccaaaaagaccaacgtcacattgagcaaaaagcgtaagcgcaggtttctgggcttcctcctgggagttggttcagctattgcgtcgggcgtagccgtgagtaaagtccttcacttggagggagaagttaataagatcaagtccgcactcctgtctactaacaaagctgtggtcagcttgtcaaacggtgtatccgtgctgacctcgaaggttcttgacctcaaaaattacatcgataagcaattgctgccgattgtcaacaagcagagttgttctatcagcaatattgagacggtgatcgagttccaacagaaaaacaacagactcctggaaatcacacgtgagttttcagtaaatgccggcgttactacccccgtctccacgtacatgcttacaaactcggaattgctcagtctgattaacgacatgcctatcactaatgatcagaagaagcttatgtctaacaacgtgcaaattgtccgccagcaaagctattccatcatgtcaatcattaaagaggaagtgttggcgtacgtagttcagctcccactgtacggagtcatcgacaccccgtgctggaagcttcatacctcgcccttgtgtacgacaaatactaaagagggttctaacatttgcctcaccaggacggatcgaggctggtattgcgataacgctggaagtgtgagcttcttccctcaagcagaaacatgtaaggtacagtccaatagagttttttgcgacactatgaactcactgacccttccatctgaggtcaatttgtgtaacgtcgatatcttcaacccgaagtacgactgcaaaattatgacgtccaagacagatgtgtcgagtagcgtaatcacttcactcggtgccatcgtttcttgctacggcaagaccaaatgtacggcttccaataagaaccgtggaattatcaaaacattctcgaacggttgcgactatgtcagcaataagggcgtggacactgtgagtgtaggaaacaccctgtactacgttaacaagcaagaaggtaaatcactgtatgtcaagggcgagcccattatcaatttttacgatcctcttgtgttcccatccgacgagttcgatgcgtctatcagccaggtaaacgaaaagattaaccagtccttggcatttatccgcaaatcggacgagctcctgcacaatgttaacgccggaaagagtacgacaaacattatgatcactaccatcattatcgtcattatcgtgatccttttgtcactcattgctgtaggtctgcttttgtactgtaaagcgaggtctacgcccgttacactcagcaaggatcaactgtccggcatcaataacattgccttctcgaattaa

SEQ ID NO: 4 - protein, 574 aa, Artificial Sequence
  F Protein 576
MELLILKANAITTILTAVTFCFASGQNITEEFYQSTCSAVSKGYLSALRTGWYTSVITIELSNIKENKCNGTDAKVKLIKQELDKYKNAVTELQLLMQSTPATNNRARRELPRFMNYTLNNAKKTNVTLSKKRKRRFLGFLLGVGSAIASGVAVSKVLHLEGEVNKIKSALLSTNKAVVSLSNGVSVLTSKVLDLKNYIDKQLLPIVNKQSCSISNIETVIEFQQKNNRLLEITREFSVNAGVTTPVSTYMLTNSELLSLINDMPITNDQKKLMSNNVQIVRQQSYSIMSIIKEEVLAYVVQLPLYGVIDTPCWKLHTSPLCTTNTKEGSNICLTRTDRGWYCDNAGSVSFFPQAETCKVQSNRVFCDTMNSLTLPSEVNLCNVDIFNPKYDCKIMTSKTDVSSSVITSLGAIVSCYGKTKCTASNKNRGIIKTFSNGCDYVSNKGVDTVSVGNTLYYVNKQEGKSLYVKGEPIINFYDPLVFPSDEFDASISQVNEKINQSLAFIRKSDELLHNVNAGKSTTNIMITTIIIVIIVILLSLIAVGLLLYCKARSTPVTLSKDQLSGINNIAFSN

SEQ ID NO: 5 - DNA, 1725 bp, Artificial Sequence
  F Protein 541
atggagctgctcatcttgaaggctaacgccattaccactatccttacagcggtgacgttctgctttgcatccggtcagaatattaccgaagagttctaccaatctacttgtagcgctgtctcaaaaggctatctgtcggccctccgtacaggatggtacacgagtgttatcaccatcgaattgtccaacattaaggagaacaagtgcaacggtactgacgcgaaggtaaagcttatcaaacaggaactggataagtacaagaacgcagtgacagagctccaattgctgatgcagtctacccccgctacgaataaccgcgctaggagagaacttccacgattcatgaactatactctcaataacgccaaaaagaccaacgtcacattgagcaaaaagcagaagcaacagtttctgggcttcctcctgggagttggttcagctattgcgtcgggcgtagccgtgagtaaagtccttcacttggagggagaagttaataagatcaagtccgcactcctgtctactaacaaagctgtggtcagcttgtcaaacggtgtatccgtgctgacctcgaaggttcttgacctcaaaaattacatcgataagcaattgctgccgattgtcaacaagcagagttgttctatcagcaatattgagacggtgatcgagttccaacagaaaaacaacagactcctggaaatcacacgtgagttttcagtaaatgccggcgttactacccccgtctccacgtacatgcttacaaactcggaattgctcagtctgattaacgacatgcctatcactaatgatcagaagaagcttatgtctaacaacgtgcaaattgtccgccagcaaagctattccatcatgtcaatcattaaagaggaagtgttggcgtacgtagttcagctcccactgtacggagtcatcgacaccccgtgctggaagcttcatacctcgcccttgtgtacgacaaatactaaagagggttctaacatttgcctcaccaggacggatcgaggctggtattgcgataacgctggaagtgtgagcttcttccctcaagcagaaacatgtaaggtacagtccaatagagttttttgcgacactatgaactcactgacccttccatctgaggtcaatttgtgtaacgtcgatatcttcaacccgaagtacgactgcaaaattatgacgtccaagacagatgtgtcgagtagcgtaatcacttcactcggtgccatcgtttcttgctacggcaagaccaaatgtacggcttccaataagaaccgtggaattatcaaaacattctcgaacggttgcgactatgtcagcaataagggcgtggacactgtgagtgtaggaaacaccctgtactacgttaacaagcaagaaggtaaatcactgtatgtcaagggcgagcccattatcaatttttacgatcctcttgtgttcccatccgacgagttcgatgcgtctatcagccaggtaaacgaaaagattaaccagtccttggcatttatccgcaaatcggacgagctcctgcacaatgttaacgccggaaagagtacgacaaacattatgatcactaccatcattatcgtcattatcgtgatccttttgtcactcattgctgtaggtctgcttttgtactgtaaagcgaggtctacgcccgttacactcagcaaggatcaactgtccggcatcaataacattgccttctcgaattaa

SEQ ID NO: 6 - protein, 574 aa, Artificial Sequence
  F protein 541
MELLILKANAITTILTAVTFCFASGQNITEEFYQSTCSAVSKGYLSALRTGWYTSVITIELSNIKENKCNGTDAKVKLIKQELDKYKNAVTELQLLMQSTPATNNRARRELPRFMNYTLNNAKKTNVTLSKKQKQQFLGFLLGVGSAIASGVAVSKVLHLEGEVNKIKSALLSTNKAVVSLSNGVSVLTSKVLDLKNYIDKQLLPIVNKQSCSISNIETVIEFQQKNNRLLEITREFSVNAGVTTPVSTYMLTNSELLSLINDMPITNDQKKLMSNNVQIVRQQSYSIMSIIKEEVLAYVVQLPLYGVIDTPCWKLHTSPLCTTNTKEGSNICLTRTDRGWYCDNAGSVSFFPQAETCKVQSNRVFCDTMNSLTLPSEVNLCNVDIFNPKYDCKIMTSKTDVSSSVITSLGAIVSCYGKTKCTASNKNRGIIKTFSNGCDYVSNKGVDTVSVGNTLYYVNKQEGKSLYVKGEPIINFYDPLVFPSDEFDASISQVNEKINQSLAFIRKSDELLHNVNAGKSTTNIMITTIIIVIIVILLSLIAVGLLLYCKARSTPVTLSKDQLSGINNIAFSN

SEQ ID NO: 7 - DNA, 1695 bp, Artificial Sequence
  F Protein 683
atggagctgctcatcttgaaggctaacgccattaccactatccttacagcggtgacgttctgctttgcatccggtcagaatattaccgaagagttctaccaatctacttgtagcgctgtctcaaaaggctatctgtcggccctccgtacaggatggtacacgagtgttatcaccatcgaattgtccaacattaaggagaacaagtgcaacggtactgacgcgaaggtaaagcttatcaaacaggaactggataagtacaagaacgcagtgacagagctccaattgctgatgcagtctacccccgctacgaataaccgcgctaggagagaacttccacgattcatgaactatactctcaataacgccaaaaagaccaacgtcacattgagcaaaaagcagaagcaacaggctattgcgtcgggcgtagccgtgagtaaagtccttcacttggagggagaagttaataagatcaagtccgcactcctgtctactaacaaagctgtggtcagcttgtcaaacggtgtatccgtgctgacctcgaaggttcttgacctcaaaaattacatcgataagcaattgctgccgattgtcaacaagcagagttgttctatcagcaatattgagacggtgatcgagttccaacagaaaaacaacagactcctggaaatcacacgtgagttttcagtaaatgccggcgttactacccccgtctccacgtacatgcttacaaactcggaattgctcagtctgattaacgacatgcctatcactaatgatcagaagaagcttatgtctaacaacgtgcaaattgtccgccagcaaagctattccatcatgtcaatcattaaagaggaagtgttggcgtacgtagttcagctcccactgtacggagtcatcgacaccccgtgctggaagcttcatacctcgcccttgtgtacgacaaatactaaagagggttctaacatttgcctcaccaggacggatcgaggctggtattgcgataacgctggaagtgtgagcttcttccctcaagcagaaacatgtaaggtacagtccaatagagttttttgcgacactatgaactcactgacccttccatctgaggtcaatttgtgtaacgtcgatatcttcaacccgaagtacgactgcaaaattatgacgtccaagacagatgtgtcgagtagcgtaatcacttcactcggtgccatcgtttcttgctacggcaagaccaaatgtacggcttccaataagaaccgtggaattatcaaaacattctcgaacggttgcgactatgtcagcaataagggcgtggacactgtgagtgtaggaaacaccctgtactacgttaacaagcaagaaggtaaatcactgtatgtcaagggcgagcccattatcaatttttacgatcctcttgtgttcccatccgacgagttcgatgcgtctatcagccaggtaaacgaaaagattaaccagtccttggcatttatccgcaaatcggacgagctcctgcacaatgttaacgccggaaagagtacgacaaacattatgatcactaccatcattatcgtcattatcgtgatccttttgtcactcattgctgtaggtctgcttttgtactgtaaagcgaggtctacgcccgttacactcagcaaggatcaactgtccggcatcaataacattgccttctcgaattaa

SEQ ID NO: 8 - protein, 564 aa, Artificial Sequence
  F protein 683
MELLILKANAITTILTAVTFCFASGQNITEEFYQSTCSAVSKGYLSALRTGWYTSVITIELSNIKENKCNGTDAKVKLIKQELDKYKNAVTELQLLMQSTPATNNRARRELPRFMNYTLNNAKKTNVTLSKKQKQQAIASGVAVSKVLHLEGEVNKIKSALLSTNKAVVSLSNGVSVLTSKVLDLKNYIDKQLLPIVNKQSCSISNIETVIEFQQKNNRLLEITREFSVNAGVTTPVSTYMLTNSELLSLINDMPITNDQKKLMSNNVQIVRQQSYSIMSIIKEEVLAYVVQLPLYGVIDTPCWKLHTSPLCTTNTKEGSNICLTRTDRGWYCDNAGSVSFFPQAETCKVQSNRVFCDTMNSLTLPSEVNLCNVDIFNPKYDCKIMTSKTDVSSSVITSLGAIVSCYGKTKCTASNKNRGIIKTFSNGCDYVSNKGVDTVSVGNTLYYVNKQEGKSLYVKGEPIINFYDPLVFPSDEFDASISQVNEKINQSLAFIRKSDELLHNVNAGKSTTNIMITTIIIVIIVILLSLIAVGLLLYCKARSTPVTLSKDQLSGINNIAFSN

SEQ ID NO: 9 - DNA, 1695 bp, Artificial Sequence
  F protein 622
atggagctgctcatcttgaaggctaacgccattaccactatccttacagcggtgacgttctgctttgcatccggtcagaatattaccgaagagttctaccaatctacttgtagcgctgtctcaaaaggctatctgtcggccctccgtacaggatggtacacgagtgttatcaccatcgaattgtccaacattaaggagaacaagtgcaacggtactgacgcgaaggtaaagcttatcaaacaggaactggataagtacaagaacgcagtgacagagctccaattgctgatgcagtctacccccgctacgaataaccgcgctaggagagaacttccacgattcatgaactatactctcaataacgccaaaaagaccaacgtcacattgagcaaaaagcgtaagcgcagggctattgcgtcgggcgtagccgtgagtaaagtccttcacttggagggagaagttaataagatcaagtccgcactcctgtctactaacaaagctgtggtcagcttgtcaaacggtgtatccgtgctgacctcgaaggttcttgacctcaaaaatcacatcgataagcaattgctgccgattgtcaacaagcagagttgttctatcagcaatattgagacggtgatcgagttccaacagaaaaacaacagactcctggaaatcacacgtgagttttcagtaaatgccggcgttactacccccgtctccacgtacatgcttacaaactcggaattgctcagtctgattaacgacatgcctatcactaatgatcagaagaagcttatgtctaacaacgtgcaaattgtccgccagcaaagctattccatcatgtcaatcattaaagaggaagtgttggcgtacgtagttcagctcccactgtacggagtcatcgacaccccgtgctggaagcttcatacctcgcccttgtgtacgacaaatactaaagagggttctaacatttgcctcaccaggacggatcgaggctggtattgcgataacgctggaagtgtgagcttcttccctcaagcagaaacatgtaaggtacagtccaatagagttttttgcgacactatgaactcactgacccttccatctgaggtcaatttgtgtaacgtcgatatcttcaacccgaagtacgactgcaaaattatgacgtccaagacagatgtgtcgagtagcgtaatcacttcactcggtgccatcgtttcttgctacggcaagaccaaatgtacggcttccaataagaaccgtggaattatcaaaacattctcgaacggttgcgactatgtcagcaataagggcgtggacactgtgagtgtaggaaacaccctgtactacgttaacaagcaagaaggtaaatcactgtatgtcaagggcgagcccattatcaatttttacgatcctcttgtgttcccatccgacgagttcgatgcgtctatcagccaggtaaacgaaaagattaaccagtccttggcatttatccgcaaatcggacgagctcctgcacaatgttaacgccggaaagagtacgacaaacattatgatcactaccatcattatcgtcattatcgtgatccttttgtcactcattgctgtaggtctgcttttgtactgtaaagcgaggtctacgcccgttacactcagcaaggatcaactgtccggcatcaataacattgccttctcgaattaa

SEQ ID NO: 10 - protein, 564 aa, Artificial Sequence
  F protein 622
MELLILKANAITTILTAVTFCFASGQNITEEFYQSTCSAVSKGYLSALRTGWYTSVITIELSNIKENKCNGTDAKVKLIKQELDKYKNAVTELQLLMQSTPATNNRARRELPRFMNYTLNNAKKTNVTLSKKRKRRAIASGVAVSKVLHLEGEVNKIKSALLSTNKAVVSLSNGVSVLTSKVLDLKNHIDKQLLPIVNKQSCSISNIETVIEFQQKNNRLLEITREFSVNAGVTTPVSTYMLTNSELLSLINDMPITNDQKKLMSNNVQIVRQQSYSIMSIIKEEVLAYVVQLPLYGVIDTPCWKLHTSPLCTTNTKEGSNICLTRTDRGWYCDNAGSVSFFPQAETCKVQSNRVFCDTMNSLTLPSEVNLCNVDIFNPKYDCKIMTSKTDVSSSVITSLGAIVSCYGKTKCTASNKNRGIIKTFSNGCDYVSNKGVDTVSVGNTLYYVNKQEGKSLYVKGEPIINFYDPLVFPSDEFDASISQVNEKINQSLAFIRKSDELLHNVNAGKSTTNIMITTIIIVIIVILLSLIAVGLLLYCKARSTPVTLSKDQLSGINNIAFSN

SEQ ID NO: 11 - DNA, 771 bp, Bovine respiratory syncytial virus
atggagacatacgtgaacaaactccatgaaggatcaacttacacagctgctgttcagtacaatgtcatagaaaaagatgatgatcctgcatctctcacaatatgggttcctatgttccaatcatccatctctgctgatttgcttataaaagaactaatcaatgtgaacatattagttcgacaaatttctactctgaaaggtccttcattgaagattatgataaactcaagaagtgctgtactagcccaaatgcccagcaaatttaccataagtgcaaatgtatcattggatgaacgaagcaaattagcatatgacataactactccttgtgaaattaaggcttgtagtttaacatgtttaaaggtgaaaaatatgctcacaactgtgaaagatctcaccatgaaaacattcaatcctacccatgagatcattgcactgtgtgaatttgaaaatatcatgacatccaaaagagttgttataccaactttcttaaggtcaatcaatgtaaaagcaaaggatttggactcactagagaatatagctaccacagagttcaaaaatgccatcactaatgctaaaattataccttatgctgggttggtattagttatcactgtaactgacaataaaggggcattcaagtacattaaaccacaaagtcaatttatagtagatcttggtgcatatctagagaaagagagcatatattatgtaactacaaattggaaacacacggccactaaattctccattaagcctatagaggactga

SEQ ID NO: 12 - protein, 256 aa, Bovine respiratory syncytial virus
METYVNKLHEGSTYTAAVQYNVIEKDDDPASLTIWVPMFQSSISADLLIKELINVNILVRQISTLKGPSLKIMINSRSAVLAQMPSKFTISANVSLDERSKLAYDITTPCEIKACSLTCLKVKNMLTTVKDLTMKTFNPTHEIIALCEFENIMTSKRVVIPTFLRSINVKAKDLDSLENIATTEFKNAITNAKIIPYAGLVLVITVTDNKGAFKYIKPQSQFIVDLGAYLEKESIYYVTTNWKHTATKFSIKPIED

SEQ ID NO: 13 - DNA, 771 bp, Artificial Sequence
  Codon Optimized Bovine RSV M
atggagacttacgtgaacaagctgcacgagggttccacctacaccgctgctgtgcagtacaacgtgatcgagaaggacgacgaccccgcttccctgaccatctgggtgcccatgttccagtcctccatctccgctgacctgctgatcaaggagctgatcaacgtcaacatcctcgtgcgtcagatctccaccctgaagggtcccagcctgaagatcatgatcaactcccgttccgctgtgctggctcagatgccctccaagttcaccatctccgccaacgtgtccctggacgagcgttccaagctggcttacgacatcaccaccccctgcgagatcaaggcttgctccctgacctgcctgaaggtcaagaacatgctgaccaccgtgaaggacctgaccatgaagaccttcaaccccacccacgagatcatcgctctgtgcgagttcgagaacatcatgacctccaagcgtgtggtcatccccaccttcctccgctccatcaacgtgaaggctaaggacctggactccctcgagaacatcgctaccaccgagttcaagaacgctatcaccaacgctaagatcatcccttacgctggcctggtgctggtcatcaccgtgaccgacaacaagggcgctttcaagtacatcaagccccagtcccagttcatcgtggacctgggcgcttacctcgagaaggagtccatctactacgtcaccaccaactggaagcacaccgctaccaagttctccatcaagcccatcgaggactaa

SEQ ID NO: 14 - protein, 256 aa, Artificial Sequence; identical to SEQ ID NO: 12
  Codon Optimized Bovine RSV M

SEQ ID NO: 15 - DNA, 1176 bp, respiratory syncytial virus
atggctcttagcaaagtcaagttgaatgatacactcaacaaagatcaacttctgtcatccagcaaatacaccatccaacggagcacaggagatagtattgatactcctaattatgatgtgcagaaacacatcaataagttatgtggcatgttattaatcacagaagatgctaatcataaattcactgggttaataggtatgttatatgcgatgtctaggttaggaagagaagacaccataaaaatactcagagatgcgggatatcatgtaaaagcaaatggagtagatgtaacaacacatcgtcaagacattaatggaaaagaaatgaaatttgaagtgttaacattggcaagcttaacaactgaaattcaaatcaacattgagatagaatctagaaaatcctacaaaaaaatgctaaaagaaatgggagaggtagctccagaatacaggcatgactctcctgattgtgggatgataatattatgtatagcagcattagtaataactaaattagcagcaggggacagatctggtcttacagccgtgattaggagagctaataatgtcctaaaaaatgaaatgaaacgttacaaaggcttactacccaaggacatagccaacagcttctatgaagtgtttgaaaaacatccccactttatagatgtttttgttcattttggtatagcacaatcttctaccagaggtggcagtagagttgaagggatttttgcaggattgtttatgaatgcctatggtgcagggcaagtgatgttacggtggggagtcttagcaaaatcagttaaaaatattatgttaggacatgctagtgtgcaagcagaaatggaacaagttgttgaggtttatgaatatgcccaaaaattgggtggtgaagcaggattctaccatatattgaacaacccaaaagcatcattattatctttgactcaatttcctcacttctccagtgtagtattaggcaatgctgctggcctaggcataatgggagagtacagaggtacaccgaggaatcaagatctatatgatgcagcaaaggcatatgctgaacaactcaaagaaaatggtgtgattaactacagtgtactagacttgacagcagaagaactagaggctatcaaacatcagcttaatccaaaagataatgatgtagagctttga

SEQ ID NO: 16 - protein, 391 aa, respiratory syncytial virus
MALSKVKLNDTLNKDQLLSSSKYTIQRSTGDSIDTPNYDVQKHINKLCGMLLITEDANHKFTGLIGMLYAMSRLGREDTIKILRDAGYHVKANGVDVTTHRQDINGKEMKFEVLTLASLTTEIQINIEIESRKSYKKMLKEMGEVAPEYRHDSPDCGMIILCIAALVITKLAAGDRSGLTAVIRRANNVLKNEMKRYKGLLPKDIANSFYEVFEKHPHFIDVFVHFGIAQSSTRGGSRVEGIFAGLFMNAYGAGQVMLRWGVLAKSVKNIMLGHASVQAEMEQVVEVYEYAQKLGGEAGFYHILNNPKASLLSLTQFPHFSSVVLGNAAGLGIMGEYRGTPRNQDLYDAAKAYAEQLKENGVINYSVLDLTAEELEAIKHQLNPKDNDVEL

SEQ ID NO: 17 - DNA, 1176 bp, Artificial Sequence
  Codon Optimized RSV N
atggctctgtccaaggtcaagctgaacgacaccctgaacaaggaccagctgctgtcctcctccaagtacaccatccagcgttccaccggtgactccatcgacacccccaactacgacgtgcagaagcacatcaacaagctgtgcggcatgctgctgatcaccgaggacgctaaccacaagttcaccggtctgatcggcatgctgtacgctatgtcccgtctgggtcgtgaggacaccatcaagatcctgcgtgacgctggttaccacgtgaaggctaacggtgtcgacgtgaccacccaccgtcaggacatcaacggcaaggagatgaagttcgaggtcctgaccctggcttccctgaccaccgagatccagatcaacatcgagatcgagtcccgtaagtcctacaagaagatgctgaaggagatgggcgaggtcgcccccgagtaccgtcacgactcccccgactgcggcatgatcatcctgtgcatcgctgctctcgtcatcaccaagctggctgctggtgaccgttccggtctgaccgctgtgatccgtcgtgctaacaacgtgctgaagaacgagatgaagcgctacaagggtctgctgcccaaggacatcgctaacagcttctacgaggtgttcgagaagcacccccacttcatcgacgtgttcgtgcacttcggtatcgctcagtcctccacccgtggtggttcccgtgtggagggcatcttcgctggtctgttcatgaacgcttacggtgctggccaggtcatgctgcgttggggtgtgctggctaagtccgtgaagaacatcatgctgggtcacgcttccgtgcaggctgagatggagcaggtggtggaggtgtacgagtacgctcagaagctgggcggcgaggctggtttctaccacatcctgaacaaccccaaggcttccctgctgtccctgacccagttcccccacttctcctccgtggtgctgggtaacgctgctggtctgggtatcatgggcgagtaccgtggcaccccccgtaaccaggacctgtacgacgctgctaaggcttacgccgagcagctcaaggagaacggcgtcatcaactactccgtgctggacctgaccgctgaggagctggaggctatcaagcaccagctgaaccccaaggacaacgacgtggagctgtaa

SEQ ID NO: 18 - protein, 391 aa, Artificial Sequence; identical to SEQ ID NO: 16
  Codon Optimized RSV N

SEQ ID NO: 19 - DNA, 1725 bp, Artificial Sequence
  F protein 368
atggagctgctcatcttgaaggctaacgccattaccactatccttacagcggtgacgttctgctttgcatccggtcagaatattaccgaagagttctaccaatctacttgtagcgctgtctcaaaaggctatctatcggccttacgtacaggatggtacacgagtgttatcaccatcgaactgtccaacattaaggagaataaatgcaacggtactgacgcgaaggtaaagctcatcaaacaggaattggataagtacaagaacgcagtgacagagcttcaactgctaatgcagtctaccccccctacgaataaccgcgctaggagagaactcccacgattcatgaactatactttaaataacgccaaaaagaccaacgtcacattgagcaaaaagcgtaagcgcaggtttctgggcttccttctcggagttggttcagctattgcgtcgggcgtagccgtgagtaaagtcttgcacctggagggagaagttaataagatcaagtccgcactcctgtctactaacaaagctgtggtcagcctatcaaacggtgtatccgtgttaacctcgaaggttcttgacttgaaaaattacatcgataagcaactcctgccgattgtcaacaagcagagttgttctatcagcaatattgagacggtgatcgagttccaacagaaaaacaacagattgctggaaatcacacgtgagttttcagtaaatgccggcgttactacccccgtctccacgtacatgctaacaaactcggaattacttagtctcattaacgacatgcctatcactaatgatcagaagaagttgatgtctaacaacgtgcaaattgtccgccagcaaagctattccatcatgtcaatcattaaagaggaagtgctggcgtacgtagttcagctcccactgtacggagtcatcgacaccccgtgctggaagctacatacctcgcccttatgtacgacaaatactaaagagggttctaacatttgccttaccaggacggatcgaggctggtattgcgataacgctggaagtgtgagcttcttccctcaagcagaaacatgtaaggtacagtccaatagagttttttgcgacactatgaactcattgaccctcccatctgagatcaatctgtgtaacgtcgatatcttcaacccgaagtacgactgcaaaattatgacgtccaagacagatgtgtcgagtagcgtaatcacttcactaggtgccatcgtttcttgctacggcaagaccaaatgtacggcttccaataagaaccgtggaattatcaaaacattctcgaacggttgcgactatgtcagcaataagggcatggacactgtgagtgtaggaaacaccttatactacgttaacaagcaagaaggtaaatcactttatgtcaagggcgagcccattatcaatttttacgatcctttggtgttcccatccgacgagttcgatgcgtctatcagccaggtaaacgaaaagattaaccagtccctcgcatttatccgcaaatcggacgagctgctacacaatgttaacgccggaaagagtacgacaaacattatgatcactaccatcattatcgtcattatcgtgatccttttgtcactcattgctgtaggtctgttactatactgtaaagcgaggtctacgcccgttacacttagcaaggatcaattgtccggcatcaataacattgccttctcgaattaa

SEQ ID NO: 20 - protein, 574 aa, Artificial Sequence; identical to SEQ ID NO: 2
  F protein 368

SEQ ID NO: 21 - protein, 560 aa, Artificial Sequence
  F protein 623
MELLILKANAITTILTAVTFCFASGQNITEEFYQSTCSAVSKGYLSALRTGWYTSVITIELSNIKENKCNGTDAKVKLIKQELDKYKNAVTELQLLMQSTPATNNRANNELPRFMNYTLNNAKKTNVTLSRRAIASGVAVSKVLHLEGEVNKIKSALLSTNKAVVSLSNGVSVLTSKVLDLKNHIDKQLLPIVNKQSCSISNIETVIEFQQKNNRLLEITREFSVNAGVTTPVSTYMLTNSELLSLINDMPITNDQKKLMSNNVQIVRQQSYSIMSIIKEEVLAYVVQLPLYGVIDTPCWKLHTSPLCTTNTKEGSNICLTRTDRGWYCDNAGSVSFFPQAETCKVQSNRVFCDTMNSLTLPSEVNLCNVDIFNPKYDCKIMTSKTDVSSSVITSLGAIVSCYGKTKCTASNKNRGIIKTFSNGCDYVSNKGVDTVSVGNTLYYVNKQEGKSLYVKGEPIINFYDPLVFPSDEFDASISQVNEKINQSLAFIRKSDELLHNVNAGKSTTNIMITTIIIVIIVILLSLIAVGLLLYCKARSTPVTLSKDQLSGINNIAFSN

SEQ ID NO: 22 - protein, 252 aa, Avian influenza virus
MSLLTEVETYVLSIIPSGPLKAEIAQKLEDVFAGKNTDLEALMEWLKTRPILSPLTKGILGFVFTLTVPSERGLQRRRFVQNALNGNGDPNNMDRAVKLYKKLKREITFHGAKEVSLSYSTGALASCMGLIYNRMGTVTTEVAFGLVCATCEQIADSQHRSHRQMATITNPLIRHENRMVLASTTAKAMEQMAGSSEQAAEAMEVANQARQMVQAMRTIGTHPNSSAGLRDNLLENLQAYQKRMGVQMQRFK

SEQ ID NO: 23 - protein, 4 aa, Artificial Sequence
  Secondary Cleavage Site
RARR

SEQ ID NO: 24 - protein, 6 aa, Artificial Sequence
  Primary Cleavage Site
KKRKRR

SEQ ID NO: 25 - DNA, 897 bp, Artificial Sequence
  Codon Optimized RSV G
atgtccaagaacaaagaccagcgtaccgctaagactctggagcgcacatgggatacgctcaatcacttgcttttcatctctagctgcctgtacaaactcaacttgaagtcagtggcccaaattaccctttcgatcctggcgatgattatcagtacttccctcatcattgcagctatcatttttatcgcctctgcgaatcataaggtcacacccacgaccgcaatcattcaggacgctactagccaaatcaaaaacacaacccctacgtatttgactcagaacccacaactgggtatttcaccgtcgaatcccagtgaaatcacctcccagatcacaactattcttgcctctaccacgcctggcgttaagagcacactccaatcaactaccgtaaagacgaaaaacacaactaccacccagacgcagccatccaagccgacaactaaacaaaggcagaacaagcccccttcgaagccaaataacgatttccacttcgaggtgtttaacttcgtcccgtgtagtatctgctctaataaccccacctgttgggctatttgcaaaagaatccctaacaagaagccaggaaaaaagacgacaactaaacccaccaagaagcctacgttgaaaacaactaagaaggacccgaaaccacaaaccacgaagagcaaagaagttcccacaactaagcctaccgaggaaccgacgatcaatacaactaagaccaacattatcacgacactgctcacttcaaataccactggtaacccagagctgacctcccagatggaaaccttccattcgacgagttctgagggcaaccccagcccttcccaagtatcaacaacttcggaatacccatctcagcccagtagccctccgaataccccacgacaataa

SEQ ID NO: 26 - protein, 298 aa, Artificial Sequence
  Codon Optimized RSV G
MSKNKDQRTAKTLERTWDTLNHLLFISSCLYKLNLKSVAQITLSILAMIISTSLIIAAIIFIASANHKVTPTTAIIQDATSQIKNTTPTYLTQNPQLGISPSNPSEITSQITTILASTTPGVKSTLQSTTVKTKNTTTTQTQPSKPTTKQRQNKPPSKPNNDFHFEVFNFVPCSICSNNPTCWAICKRIPNKKPGKKTTTKPTKKPTLKTTKKDPKPQTTKSKEVPTTKPTEEPTINTTKTNIITTLLTSNTTGNPELTSQMETFHSTSSEGNPSPSQVSTTSEYPSQPSSPPNTPRQ

SEQ ID NO: 27 - protein, 65 aa, respiratory syncytial virus
MGNTSITIEFTSKFWPYFTLIHMILTLISLLIIITIMIAILNKLSEHKTFCNNTLELGQMHQINT

SEQ ID NO: 28 - protein, 6 aa, Artificial Sequence
  Furin Recognition Site Mutation
KKQKQQ

SEQ ID NO: 29 - protein, 6 aa, Artificial Sequence
  Furin Recognition Site Mutation
GRRQQR